European Patent Specification EP 3 784 255 B1, published September 17, 2025. Title: T CELL RECEPTORS WITH MAGE-B2 SPECIFICITY AND USES THEREOF. Applicant: The Board of Regents of the University of Texas. The sequence listing filed with the application follows.

SEQUENCE LISTING (45 sequences)

SEQ ID NO: 1 - protein, 10 aa, Artificial sequence
  Synthetic amino acid
GVYDGEEHSV

SEQ ID NO: 2 - DNA, 813 bp, Artificial sequence
  Synthetic oligonucleotide
atgaactattctccaggcttagtatctctgatactcttactgcttggaagaacccgtggaaattcagtgacccagatggaagggccagtgactctctcagaagaggccttcctgactataaactgcacgtacacagccacaggatacccttcccttttctggtatgtccaatatcctggagaaggtctacagctcctcctgaaagccacgaaggctgatgacaagggaagcaacaaaggttttgaagccacataccgtaaagaaaccacttctttccacttggagaaaggctcagttcaagtgtcagactcagcggtgtacttctgtgctctgaccaacgactacaagctcagctttggagccggaaccacagtaactgtaagagcaaatatccagaaccctgaccctgccgtgtaccagctgagagactctaaatccagtgacaagtctgtctgcctattcaccgattttgattctcaaacaaatgtgtcacaaagtaaggattctgatgtgtatatcacagacaaaactgtgctagacatgaggtctatggacttcaagagcaacagtgctgtggcctggagcaacaaatctgactttgcatgtgcaaacgccttcaacaacagcattattccagaagacaccttcttccccagcccagaaagttcctgtgatgtcaagctggtcgagaaaagctttgaaacagatacgaacctaaactttcaaaacctgtcagtgattgggttccgaatcctcctcctgaaagtggccgggtttaatctgctcatgacgctgcggctgtggtccagctga

SEQ ID NO: 3 - protein, 220 aa, Artificial sequence
  Synthetic amino acid
SLFWYVQYPGEGLQLLLKATKADDKGSNKGFEATYRKETTSFHLEKGSVQVSDSAVYFCALTNDYKLSFGAGTTVTVRANIQNPDPAVYQLRDSKSSDKSVCLFTDFDSQTNVSQSKDSDVYITDKTVLDMRSMDFKSNSAVAWSNKSDFACANAFNNSIIPEDTFFPSPESSCDVKLVEKSFETDTNLNFQNLSVIGFRILLLKVAGFNLLMTLRLWSS

SEQ ID NO: 4 - DNA, 930 bp, Artificial sequence
  Synthetic oligonucleotide
atgggtcctgggcttctccactggatggccctttgtctccttggaacaggtcatggggatgccatggtcatccagaacccaagataccaggttacccagtttggaaagccagtgaccctgagttgttctcagactttgaaccataacgtcatgtactggtaccagcagaagtcaagtcaggccccaaagctgctgttccactactatgacaaagattttaacaatgaagcagacacccctgataacttccaatccaggaggccgaacacttctttctgctttcttgacatccgctcaccaggcctgggggacgcagccatgtacctgtgtgccaccagcaggggcgggaggtacaatgagcagttcttcgggccagggacacggctcaccgtgctagaggacctgaaaaacgtgttcccacccgaggtcgctgtgtttgagccatcagaagcagagatctcccacacccaaaaggccacactggtgtgcctggccacaggcttcttccctgaccacgtggagctgagctggtgggtgaatgggaaggaggtgcacagtggggtcagcacggacccgcagcccctcaaggagcagcccgccctcaatgactccagatactgcctgagcagccgcctgagggtctcggccaccttctggcagaacccccgcaaccacttccgctgtcaagtccagttctacgggctctcggagaatgacgagtggacccaggatagggccaaacccgtcacccagatcgtcagcgccgaggcctggggtagagcagactgtggctttacctcggtgtcctaccagcaaggggtcctgtctgccaccatcctctatgagatcctgctagggaaggccaccctgtatgctgtgctggtcagcgcccttgtgttgatggccatggtcaagagaaaggatttctga

SEQ ID NO: 5 - protein, 309 aa, Artificial sequence
  Synthetic amino acid
MGPGLLHWMALCLLGTGHGDAMVIQNPRYQVTQFGKPVTLSCSQTLNHNVMYWYQQKSSQAPKLLFHYYDKDFNNEADTPDNFQSRRPNTSFCFLDIRSPGLGDAAMYLCATSRGGRYNEQFFGPGTRLTVLEDLKNVFPPEVAVFEPSEAEISHTQKATLVCLATGFFPDHVELSWWVNGKEVHSGVSTDPQPLKEQPALNDSRYCLSSRLRVSATFWQNPRNHFRCQVQFYGLSENDEWTQDRAKPVTQIVSAEAWGRADCGFTSVSYQQGVLSATILYEILLGKATLYAVLVSALVLMAMVKRKDF

SEQ ID NO: 6 - DNA, 18 bp, Artificial sequence
  Synthetic oligonucleotide
gccacaggatacccttcc

SEQ ID NO: 7 - protein, 6 aa, Artificial sequence
  Synthetic amino acid
ATGYPS

SEQ ID NO: 8 - DNA, 21 bp, Artificial sequence
  Synthetic oligonucleotide
gccacgaaggctgatgacaag

SEQ ID NO: 9 - protein, 7 aa, Artificial sequence
  Synthetic amino acid
ATKADDK

SEQ ID NO: 10 - DNA, 27 bp, Artificial sequence
  Synthetic oligonucleotide
gctctgaccaacgactacaagctcagc

SEQ ID NO: 11 - protein, 9 aa, Artificial sequence
  Synthetic amino acid
ALTNDYKLS

SEQ ID NO: 12 - DNA, 15 bp, Artificial sequence
  Synthetic oligonucleotide
ttgaaccataacgtc

SEQ ID NO: 13 - protein, 5 aa, Artificial sequence
  Synthetic amino acid
LNHNV

SEQ ID NO: 14 - DNA, 18 bp, Artificial sequence
  Synthetic oligonucleotide
tactatgacaaagatttt

SEQ ID NO: 15 - protein, 6 aa, Artificial sequence
  Synthetic amino acid
YYDKDF

SEQ ID NO: 16 - DNA, 36 bp, Artificial sequence
  Synthetic oligonucleotide
gccaccagcaggggcgggaggtacaatgagcagttc

SEQ ID NO: 17 - protein, 12 aa, Artificial sequence
  Synthetic amino acid
ATSRGGRYNEQF

SEQ ID NO: 18 - DNA, 822 bp, Artificial Sequence
  Alpha Chain (TRAV10*01)
atgaaaaagcatctgacgaccttcttggtgattttgtggctttatttttatagggggaatggcaaaaaccaagtggagcagagtcctcagtccctgatcatcctggagggaaagaactgcactcttcaatgcaattatacagtgagccccttcagcaacttaaggtggtataagcaagatactgggagaggtcctgtttccctgacaatcatgactttcagtgagaacacaaagtcgaacggaagatatacagcaactctggatgcagacacaaagcaaagctctctgcacatcacagcctcccagctcagcgattcagcctcctacatctgtgtggtgatttcaggctttcagaaacttgtatttggaactggcacccgacttctggtcagtccaaatatccagaaccctgaccctgccgtgtaccagctgagagactctaaatccagtgacaagtctgtctgcctattcaccgattttgattctcaaacaaatgtgtcacaaagtaaggattctgatgtgtatatcacagacaaaactgtgctagacatgaggtctatggacttcaagagcaacagtgctgtggcctggagcaacaaatctgactttgcatgtgcaaacgccttcaacaacagcattattccagaagacaccttcttccccagcccagaaagttcctgtgatgtcaagctggtcgagaaaagctttgaaacagatacgaacctaaactttcaaaacctgtcagtgattgggttccgaatcctcctcctgaaagtggccgggtttaatctgctcatgacgctgcggctgtggtccagctaa

SEQ ID NO: 19 - protein, 273 aa, Artificial Sequence
  Alpha Chain
MKKHLTTFLVILWLYFYRGNGKNQVEQSPQSLIILEGKNCTLQCNYTVSPFSNLRWYKQDTGRGPVSLTIMTFSENTKSNGRYTATLDADTKQSSLHITASQLSDSASYICVVISGFQKLVFGTGTRLLVSPNIQNPDPAVYQLRDSKSSDKSVCLFTDFDSQTNVSQSKDSDVYITDKTVLDMRSMDFKSNSAVAWSNKSDFACANAFNNSIIPEDTFFPSPESSCDVKLVEKSFETDTNLNFQNLSVIGFRILLLKVAGFNLLMTLRLWSS

SEQ ID NO: 20 - DNA, 939 bp, Artificial Sequence
  Beta Chain (TRBV11-3*04)
atgggtaccaggctcctctgctgggtggccttctgtctcctggtggaagaactcatagaagctggagtggttcagtctcccagatataagattatagagaaaaaacagcctgtggctttttggtgcaatcctatttctggccacaataccctttactggtaccggcagaacttgggacagggcccggagcttctgattcgatatgagaatgaggaagcagtagacgattcacagttgcctaaggatcgattttctgcagagaggctcaaaggagtagactccactctcaagatccagcctgcagagcttggggactcggccgtgtatctctgtgccagcagcttccctaaacagggatcctacaatgagcagttcttcgggccagggacacggctcaccgtgctagaggacctgaaaaacgtgttcccacccgaggtcgctgtgtttgagccatcagaagcagagatctcccacacccaaaaggccacactggtgtgcctggccacaggcttcttccctgaccacgtggagctgagctggtgggtgaatgggaaggaggtgcacagtggggtcagcacggacccgcagcccctcaaggagcagcccgccctcaatgactccagatactgcctgagcagccgcctgagggtctcggccaccttctggcagaacccccgcaaccacttccgctgtcaagtccagttctacgggctctcggagaatgacgagtggacccaggatagggccaaacccgtcacccagatcgtcagcgccgaggcctggggtagagcagactgtggctttacctcggtgtcctaccagcaaggggtcctgtctgccaccatcctctatgagatcctgctagggaaggccaccctgtatgctgtgctggtcagcgcccttgtgttgatggccatggtcaagagaaaggatttctaa

SEQ ID NO: 21 - protein, 312 aa, Artificial Sequence
  Beta Chain
MGTRLLCWVAFCLLVEELIEAGVVQSPRYKIIEKKQPVAFWCNPISGHNTLYWYRQNLGQGPELLIRYENEEAVDDSQLPKDRFSAERLKGVDSTLKIQPAELGDSAVYLCASSFPKQGSYNEQFFGPGTRLTVLEDLKNVFPPEVAVFEPSEAEISHTQKATLVCLATGFFPDHVELSWWVNGKEVHSGVSTDPQPLKEQPALNDSRYCLSSRLRVSATFWQNPRNHFRCQVQFYGLSENDEWTQDRAKPVTQIVSAEAWGRADCGFTSVSYQQGVLSATILYEILLGKATLYAVLVSALVLMAMVKRKDF

SEQ ID NO: 22 - DNA, 18 bp, Artificial Sequence
  Alpha Chain CDR1
gtgagccccttcagcaac

SEQ ID NO: 23 - protein, 6 aa, Artificial Sequence
  Alpha chain CDR1
VSPFSN

SEQ ID NO: 24 - DNA, 21 bp, Artificial Sequence
  Alpha chain CDR2
atgactttcagtgagaacaca

SEQ ID NO: 25 - protein, 7 aa, Artificial Sequence
  Alpha chain CDR2
MTFSENT

SEQ ID NO: 26 - DNA, 30 bp, Artificial Sequence
  Alpha chai CDR3
gtggtgatttcaggctttcagaaacttgta

SEQ ID NO: 27 - protein, 10 aa, Artificial Sequence
  Alpha chain CDR3
VVISGFQKLV

SEQ ID NO: 28 - DNA, 15 bp, Artificial Sequence
  Beta chain CDR1
tctggccacaatacc

SEQ ID NO: 29 - protein, 5 aa, Artificial Sequence
  Beta chain CDR1
SGHNT

SEQ ID NO: 30 - DNA, 18 bp, Artificial Sequence
  Beta chain CDR2
tatgagaatgaggaagca

SEQ ID NO: 31 - protein, 6 aa, Artificial Sequence
  Beta hain CDR2
YENEEA

SEQ ID NO: 32 - DNA, 42 bp, Artificial Sequence
  Beta chain CDR3
gccagcagcttccctaaacagggatcctacaatgagcagttc

SEQ ID NO: 33 - protein, 14 aa, Artificial Sequence
  Beta chain CDR3
ASSFPKQGSYNEQF

SEQ ID NO: 34 - DNA, 57 bp, Artificial Sequence
  Alpha chain signal peptide
atgaactattctccaggcttagtatctctgatactcttactgcttggaagaacccgt

SEQ ID NO: 35 - protein, 19 aa, Artificial Sequence
  Alpha chain signal peptide 3
MNYSPGLVSLILLLLGRTR

SEQ ID NO: 36 - DNA, 336 bp, Artificial Sequence
  Alpha chain variable region 2
ggaaattcagtgacccagatggaagggccagtgactctctcagaagaggccttcctgactataaactgcacgtacacagccacaggatacccttcccttttctggtatgtccaatatcctggagaaggtctacagctcctcctgaaagccacgaaggctgatgacaagggaagcaacaaaggttttgaagccacataccgtaaagaaaccacttctttccacttggagaaaggctcagttcaagtgtcagactcagcggtgtacttctgtgctctgaccaacgactacaagctcagctttggagccggaaccacagtaactgtaagagcaaatatc

SEQ ID NO: 37 - protein, 111 aa, Artificial Sequence
  Alpha chain variable region 3
GNSVTQMEGPVTLSEEAFLTINCTYTATGYPSLFWYVQYPGEGLQLLLKATKADDKGSNKGFEATYRKETTSFHLEKGSVQVSDSAVYFCALTNDYKLSFGAGTTVTVRAN

SEQ ID NO: 38 - DNA, 420 bp, Artificial Sequence
  Alpha chain constant region 2
cagaaccctgaccctgccgtgtaccagctgagagactctaaatccagtgacaagtctgtctgcctattcaccgattttgattctcaaacaaatgtgtcacaaagtaaggattctgatgtgtatatcacagacaaaactgtgctagacatgaggtctatggacttcaagagcaacagtgctgtggcctggagcaacaaatctgactttgcatgtgcaaacgccttcaacaacagcattattccagaagacaccttcttccccagcccagaaagttcctgtgatgtcaagctggtcgagaaaagctttgaaacagatacgaacctaaactttcaaaacctgtcagtgattgggttccgaatcctcctcctgaaagtggccgggtttaatctgctcatgacgctgcggctgtggtccagctga

SEQ ID NO: 39 - protein, 140 aa, Artificial Sequence
  Alpha chain constant region 3
IQNPDPAVYQLRDSKSSDKSVCLFTDFDSQTNVSQSKDSDVYITDKTVLDMRSMDFKSNSAVAWSNKSDFACANAFNNSIIPEDTFFPSPESSCDVKLVEKSFETDTNLNFQNLSVIGFRILLLKVAGFNLLMTLRLWSS

SEQ ID NO: 40 - DNA, 57 bp, Artificial Sequence
  Beta chain signal peptide 4
atgggtcctgggcttctccactggatggccctttgtctccttggaacaggtcatggg

SEQ ID NO: 41 - protein, 19 aa, Artificial Sequence
  Beta chain signal peptide 5
MGPGLLHWMALCLLGTGHG

SEQ ID NO: 42 - DNA, 342 bp, Artificial Sequence
  Beta chain variable region 4
gatgccatggtcatccagaacccaagataccaggttacccagtttggaaagccagtgaccctgagttgttctcagactttgaaccataacgtcatgtactggtaccagcagaagtcaagtcaggccccaaagctgctgttccactactatgacaaagattttaacaatgaagcagacacccctgataacttccaatccaggaggccgaacacttctttctgctttcttgacatccgctcaccaggcctgggggacgcagccatgtacctgtgtgccaccagcaggggcgggaggtacaatgagcagttcttcgggccagggacacggctcaccgtgctagag

SEQ ID NO: 43 - protein, 114 aa, Artificial Sequence
  Beta chain variable region 5
DAMVIQNPRYQVTQFGKPVTLSCSQTLNHNVMYWYQQKSSQAPKLLFHYYDKDFNNEADTPDNFQSRRPNTSFCFLDIRSPGLGDAAMYLCATSRGGRYNEQFFGPGTRLTVLE

SEQ ID NO: 44 - DNA, 531 bp, Artificial Sequence
  Beta chain constant region 4
gacctgaaaaacgtgttcccacccgaggtcgctgtgtttgagccatcagaagcagagatctcccacacccaaaaggccacactggtgtgcctggccacaggcttcttccctgaccacgtggagctgagctggtgggtgaatgggaaggaggtgcacagtggggtcagcacggacccgcagcccctcaaggagcagcccgccctcaatgactccagatactgcctgagcagccgcctgagggtctcggccaccttctggcagaacccccgcaaccacttccgctgtcaagtccagttctacgggctctcggagaatgacgagtggacccaggatagggccaaacccgtcacccagatcgtcagcgccgaggcctggggtagagcagactgtggctttacctcggtgtcctaccagcaaggggtcctgtctgccaccatcctctatgagatcctgctagggaaggccaccctgtatgctgtgctggtcagcgcccttgtgttgatggccatggtcaagagaaaggatttctga

SEQ ID NO: 45 - protein, 175 aa, Artificial Sequence
  Beta chain constant region 5
DLKNVFPPEVAVFEPSEAEISHTQKATLVCLATGFFPDHVELSWWVNGKEVHSGVSTDPQPLKEQPALNDSRYCLSSRLRVSATFWQNPRNHFRCQVQFYGLSENDEWTQDRAKPVTQIVSAEAWGRADCGFTSVSYQQGVLSATILYEILLGKATLYAVLVSALVLMAMVKRKD